European Patent Application EP 4 600 363 A1, published August 13, 2025. Title: A novel polynucleotide and method for producing L-alanine using thereof. Applicant: CJ CheilJedang Corporation. Application KR. The sequence listing filed with the application follows.

SEQUENCE LISTING (8 sequences)

SEQ ID NO: 1 - DNA, 100 bp, synthetic construct
  misc_feature 1..100: note = avtA promoter region_mutant
  source 1..100: mol_type = other DNA
gctgcattagagggtcgtatctcgatctaaaagcagtacgcagatataattgtctcttatgaagccaagcactagaagcaatgttcagccgtttcgcgtc

SEQ ID NO: 2 - DNA, 100 bp, synthetic construct
  misc_feature 1..100: note = avtA promoter region_wt
  source 1..100: mol_type = other DNA
gctgcattagagggtcgtatctcgatctaaaagcagtacgcagataggcttgtctcttatgaagccaagcactagaagcaatgttcagccgtttcgcgtc

SEQ ID NO: 3 - DNA, 36 bp, synthetic construct
  misc_feature 1..36: note = Pm_avtA_AF
  source 1..36: mol_type = other DNA
ctcggtacccggggatccgtctgctttatgcaggta

SEQ ID NO: 4 - DNA, 26 bp, synthetic construct
  misc_feature 1..26: note = Pm_avtA_AR
  source 1..26: mol_type = other DNA
aagagacaattatatctgcgtactgc

SEQ ID NO: 5 - DNA, 25 bp, synthetic construct
  misc_feature 1..25: note = Pm_avtA_BF
  source 1..25: mol_type = other DNA
agcagtacgcagatataattgtctc

SEQ ID NO: 6 - DNA, 36 bp, synthetic construct
  misc_feature 1..36: note = Pm_avtA_BR
  source 1..36: mol_type = other DNA
gcatgcctgcaggtcgacgtacttggacaaggtacc

SEQ ID NO: 7 - DNA, 21 bp, synthetic construct
  misc_feature 1..21: note = avtA_CF
  source 1..21: mol_type = other DNA
cgtacaccaccatcaaggaca

SEQ ID NO: 8 - DNA, 21 bp, synthetic construct
  misc_feature 1..21: note = avtA_CR
  source 1..21: mol_type = other DNA
caaaggacccgagcgaagagc